European Patent Application EP 4 230 748 A1, published August 23, 2023. Title: GENERATION OF DOUBLE-STRANDED DNA TEMPLATES FOR SINGLE MOLECULE SEQUENCING. Applicant: F. Hoffmann-La Roche AG. Application EP 19708494.0. The sequence listing filed with the application follows.

SEQUENCE LISTING (2 sequences)

SEQ ID NO: 1 - DNA, 36 bp, synthetic construct
  source 1..36: mol_type = other DNA
atctctctctactgactgtcctcctcctccgttttt

SEQ ID NO: 2 - DNA, 10 bp, synthetic construct
  source 1..10: mol_type = other DNA
gagagagatt